European Patent Application EP 4 744 659 A1, published May 20, 2026. Title: 一种抗体衍生物及其应用. Applicant: 清华大学. The sequence listing filed with the application follows.

SEQUENCE LISTING (285 sequences)

SEQ ID NO: 1 - protein, 7 aa, synthetic construct
LVPRGSG

SEQ ID NO: 2 - protein, 10 aa, synthetic construct
NSLGSQHQAQ

SEQ ID NO: 3 - protein, 12 aa, synthetic construct
GGSHHTDLPGGS

SEQ ID NO: 4 - protein, 7 aa, synthetic construct
PGSHHWG

SEQ ID NO: 5 - protein, 9 aa, synthetic construct
  SITE 3: note = natural amino acid or unnatural amino acid
QQXYTTPPT

SEQ ID NO: 6 - protein, 10 aa, synthetic construct
  SITE 4: note = natural amino acid or unnatural amino acid
CQQXYTTPPT

SEQ ID NO: 7 - protein, 11 aa, synthetic construct
  SITE 5: note = natural amino acid or unnatural amino acid
YCQQXYTTPPT

SEQ ID NO: 8 - protein, 12 aa, synthetic construct
  SITE 6: note = natural amino acid or unnatural amino acid
YYCQQXYTTPPT

SEQ ID NO: 9 - protein, 13 aa, synthetic construct
  SITE 7: note = natural amino acid or unnatural amino acid
TYYCQQXYTTPPT

SEQ ID NO: 10 - protein, 10 aa, synthetic construct
  SITE 3: note = natural amino acid or unnatural amino acid
QQXYTTPPTF

SEQ ID NO: 11 - protein, 11 aa, synthetic construct
  SITE 3: note = natural amino acid or unnatural amino acid
QQXYTTPPTFG

SEQ ID NO: 12 - protein, 12 aa, synthetic construct
  SITE 3: note = natural amino acid or unnatural amino acid
QQXYTTPPTFGQ

SEQ ID NO: 13 - protein, 13 aa, synthetic construct
  SITE 3: note = natural amino acid or unnatural amino acid
QQXYTTPPTFGQG

SEQ ID NO: 14 - protein, 11 aa, synthetic construct
  SITE 4: note = natural amino acid or unnatural amino acid
CQQXYTTPPTF

SEQ ID NO: 15 - protein, 12 aa, synthetic construct
  SITE 4: note = natural amino acid or unnatural amino acid
CQQXYTTPPTFG

SEQ ID NO: 16 - protein, 13 aa, synthetic construct
  SITE 4: note = natural amino acid or unnatural amino acid
CQQXYTTPPTFGQ

SEQ ID NO: 17 - protein, 14 aa, synthetic construct
  SITE 4: note = natural amino acid or unnatural amino acid
CQQXYTTPPTFGQG

SEQ ID NO: 18 - protein, 12 aa, synthetic construct
  SITE 5: note = natural amino acid or unnatural amino acid
YCQQXYTTPPTF

SEQ ID NO: 19 - protein, 13 aa, synthetic construct
  SITE 5: note = natural amino acid or unnatural amino acid
YCQQXYTTPPTFG

SEQ ID NO: 20 - protein, 14 aa, synthetic construct
  SITE 5: note = natural amino acid or unnatural amino acid
YCQQXYTTPPTFGQ

SEQ ID NO: 21 - protein, 15 aa, synthetic construct
  SITE 5: note = natural amino acid or unnatural amino acid
YCQQXYTTPPTFGQG

SEQ ID NO: 22 - protein, 13 aa, synthetic construct
  SITE 6: note = natural amino acid or unnatural amino acid
YYCQQXYTTPPTF

SEQ ID NO: 23 - protein, 14 aa, synthetic construct
  SITE 6: note = natural amino acid or unnatural amino acid
YYCQQXYTTPPTFG

SEQ ID NO: 24 - protein, 15 aa, synthetic construct
  SITE 6: note = natural amino acid or unnatural amino acid
YYCQQXYTTPPTFGQ

SEQ ID NO: 25 - protein, 16 aa, synthetic construct
  SITE 6: note = natural amino acid or unnatural amino acid
YYCQQXYTTPPTFGQG

SEQ ID NO: 26 - protein, 14 aa, synthetic construct
  SITE 7: note = natural amino acid or unnatural amino acid
TYYCQQXYTTPPTF

SEQ ID NO: 27 - protein, 15 aa, synthetic construct
  SITE 7: note = natural amino acid or unnatural amino acid
TYYCQQXYTTPPTFG

SEQ ID NO: 28 - protein, 16 aa, synthetic construct
  SITE 7: note = natural amino acid or unnatural amino acid
TYYCQQXYTTPPTFGQ

SEQ ID NO: 29 - protein, 17 aa, synthetic construct
  SITE 7: note = natural amino acid or unnatural amino acid
TYYCQQXYTTPPTFGQG

SEQ ID NO: 30 - protein, 11 aa, synthetic construct
RASQSISSWLA

SEQ ID NO: 31 - protein, 11 aa, synthetic construct
RASQGISRWLA

SEQ ID NO: 32 - protein, 11 aa, synthetic construct
RATQAISNYLA

SEQ ID NO: 33 - protein, 11 aa, synthetic construct
RTSQGITDPLN

SEQ ID NO: 34 - protein, 11 aa, synthetic construct
RASQGLSSWLA

SEQ ID NO: 35 - protein, 11 aa, synthetic construct
RASQNIGTYLA

SEQ ID NO: 36 - protein, 11 aa, synthetic construct
RASQGINNYLA

SEQ ID NO: 37 - protein, 11 aa, synthetic construct
QASHDISKYLN

SEQ ID NO: 38 - protein, 11 aa, synthetic construct
RASETIGSWLA

SEQ ID NO: 39 - protein, 11 aa, synthetic construct
QASQDISNYLN

SEQ ID NO: 40 - protein, 16 aa, synthetic construct
KLLIYDVSNVQTGVPS

SEQ ID NO: 41 - protein, 16 aa, synthetic construct
NLLIYGASTLQSGVPP

SEQ ID NO: 42 - protein, 16 aa, synthetic construct
KLLIYKTSSLESGVPS

SEQ ID NO: 43 - protein, 16 aa, synthetic construct
KLLIYDASNLETGVPS

SEQ ID NO: 44 - protein, 16 aa, synthetic construct
NLLIYAASTLQSGVSS

SEQ ID NO: 45 - protein, 16 aa, synthetic construct
NLLIYAASTLQSGVPS

SEQ ID NO: 46 - protein, 9 aa, synthetic construct
FTLSTYAMH

SEQ ID NO: 47 - protein, 9 aa, synthetic construct
FTFSSYWMH

SEQ ID NO: 48 - protein, 9 aa, synthetic construct
ITFGSYTMS

SEQ ID NO: 49 - protein, 9 aa, synthetic construct
FTFSSYWMN

SEQ ID NO: 50 - protein, 9 aa, synthetic construct
FTFSNYAMH

SEQ ID NO: 51 - protein, 9 aa, synthetic construct
FTFSHYAMH

SEQ ID NO: 52 - protein, 9 aa, synthetic construct
FTFSGHWMH

SEQ ID NO: 53 - protein, 9 aa, synthetic construct
FAFSSYSMS

SEQ ID NO: 54 - protein, 9 aa, synthetic construct
FTFSTYAIH

SEQ ID NO: 55 - protein, 9 aa, synthetic construct
FTFSSYGMH

SEQ ID NO: 56 - protein, 21 aa, synthetic construct
WLARIDWDDDKYYSTSLKTRL

SEQ ID NO: 57 - protein, 22 aa, synthetic construct
WVSAVSGSGDSTYYADSVKGRF

SEQ ID NO: 58 - protein, 21 aa, synthetic construct
WIGTVHYTGKTFYSPSLKSRV

SEQ ID NO: 59 - protein, 22 aa, synthetic construct
WVANIKQDGSEKYYVDSVKGRF

SEQ ID NO: 60 - protein, 22 aa, synthetic construct
WVSAISGSGGSTYYADSVKGRF

SEQ ID NO: 61 - protein, 21 aa, synthetic construct
WIGNIYYSGSTYYNPSLKSRV

SEQ ID NO: 62 - protein, 21 aa, synthetic construct
WIGSIYYSGSTYYNPSLKSRV

SEQ ID NO: 63 - protein, 24 aa, synthetic construct
WVSSISGSGGGGGTYYADSVKGRF

SEQ ID NO: 64 - protein, 22 aa, synthetic construct
WVAAISYDGSNELYADSVKGRF

SEQ ID NO: 65 - protein, 17 aa, synthetic construct
ARGRDFGEPPYVRAFDI

SEQ ID NO: 66 - protein, 10 aa, synthetic construct
AREGDWGLDY

SEQ ID NO: 67 - protein, 9 aa, synthetic construct
VTGSYRYAY

SEQ ID NO: 68 - protein, 11 aa, synthetic construct
ARGGGNYYDDY

SEQ ID NO: 69 - protein, 16 aa, synthetic construct
AKGHGSGSYFPYYFDY

SEQ ID NO: 70 - protein, 11 aa, synthetic construct
ARDRGWLQFDY

SEQ ID NO: 71 - protein, 11 aa, synthetic construct
ARNSGFETLDY

SEQ ID NO: 72 - protein, 11 aa, synthetic construct
ARDRGFLQFDY

SEQ ID NO: 73 - protein, 117 aa, synthetic construct
EVQLVESGGGLVQPGGSLRLSCAASGFAFSSYSMSWVRQAPGKGLEWIGSIYYSGSTYYNPSLKSRVTISADTSKNTAYLQMNSLRAEDTAVYYCARNSGFETLDYWGQGTLVTVSS

SEQ ID NO: 74 - protein, 120 aa, synthetic construct
EVQLVESGGGLVQPGGSLRLSCAASGFTFSTYAIHWVRQAPGKGLEWVSSISGSGGGGGTYYADSVKGRFTISADTSKNTAYLQMNSLRAEDTAVYYCARDRGFLQFDYWGQGTLVTVSS

SEQ ID NO: 75 - protein, 123 aa, synthetic construct
EVQLVESGGGLVQPGGSLRLSCAASGFTLSTYAMHWVRQAPGKGLEWLARIDWDDDKYYSTSLKTRLTISADTSKNTAYLQMNSLRAEDTAVYYCARGRDFGEPPYVRAFDIWGQGTLVTVSS

SEQ ID NO: 76 - protein, 117 aa, synthetic construct
EVQLVESGGGLVQPGGSLRLSCAASGFTFSSYWMHWVRQAPGKGLEWVSAVSGSGDSTYYADSVKGRFTISADTSKNTAYLQMNSLRAEDTAVYYCAREGDWGLDYWGQGTLVTVSS

SEQ ID NO: 77 - protein, 123 aa, synthetic construct
EVQLVESGGGLVQPGGSLRLSCAASGITFGSYTMSWVRQAPGKGLEWIGTVHYTGKTFYSPSLKSRVTISADTSKNTAYLQMNSLRAEDTAVYYCARGRDFGEPPYVRAFDIWGQGTLVTVSS

SEQ ID NO: 78 - protein, 116 aa, synthetic construct
EVQLVESGGGLVQPGGSLRLSCAASGFTFSSYWMNWVRQAPGKGLEWVANIKQDGSEKYYVDSVKGRFTISADTSKNTAYLQMNSLRAEDTAVYYCVTGSYRYAYWGQGTLVTVSS

SEQ ID NO: 79 - protein, 118 aa, synthetic construct
EVQLVESGGGLVQPGGSLRLSCAASGFTFSNYAMHWVRQAPGKGLEWVSAISGSGGSTYYADSVKGRFTISADTSKNTAYLQMNSLRAEDTAVYYCARGGGNYYDDYWGQGTLVTVSS

SEQ ID NO: 80 - protein, 122 aa, synthetic construct
EVQLVESGGGLVQPGGSLRLSCAASGFTFSHYAMHWVRQAPGKGLEWIGNIYYSGSTYYNPSLKSRVTISADTSKNTAYLQMNSLRAEDTAVYYCAKGHGSGSYFPYYFDYWGQGTLVTVSS

SEQ ID NO: 81 - protein, 117 aa, synthetic construct
EVQLVESGGGLVQPGGSLRLSCAASGFTFSGHWMHWVRQAPGKGLEWIGSIYYSGSTYYNPSLKSRVTISADTSKNTAYLQMNSLRAEDTAVYYCARDRGWLQFDYWGQGTLVTVSS

SEQ ID NO: 82 - protein, 118 aa, synthetic construct
EVQLVESGGGLVQPGGSLRLSCAASGFTFSSYGMHWVRQAPGKGLEWVAAISYDGSNELYADSVKGRFTISADTSKNTAYLQMNSLRAEDTAVYYCARDRGWLQFDYWGQGTLVTVSS

SEQ ID NO: 83 - protein, 106 aa, synthetic construct
  SITE 91: note = natural amino acid or unnatural amino acid
DIQMTQSPSSLSASVGDRVTITCRASQGISRWLAWYQQKPGKAPNLLIYGASTLQSGVPPRFSGSRSGTDFTLTISSLQPEDFATYYCQQXYTTPPTFGQGTKLEI

SEQ ID NO: 84 - protein, 106 aa, synthetic construct
  SITE 91: note = natural amino acid or unnatural amino acid
DIQMTQSPSSLSASVGDRVTITCRASQSISSWLAWYQQKPGKAPKLLIYDVSNVQTGVPSRFSGSRSGTDFTLTISSLQPEDFATYYCQQXYTTPPTFGQGTKLEI

SEQ ID NO: 85 - protein, 106 aa, synthetic construct
  SITE 91: note = natural amino acid or unnatural amino acid
DIQMTQSPSSLSASVGDRVTITCRASETIGSWLAWYQQKPGKAPNLLIYAASTLQSGVSSRFSGSRSGTDFTLTISSLQPEDFATYYCQQXYTTPPTFGQGTKLEI

SEQ ID NO: 86 - protein, 106 aa, synthetic construct
  SITE 91: note = natural amino acid or unnatural amino acid
DIQMTQSPSSLSASVGDRVTITCRASQGINNYLAWYQQKPGKAPKLLIYDASNLETGVPSRFSGSRSGTDFTLTISSLQPEDFATYYCQQXYTTPPTFGQGTKLEI

SEQ ID NO: 87 - protein, 106 aa, synthetic construct
  SITE 91: note = natural amino acid or unnatural amino acid
DIQMTQSPSSLSASVGDRVTITCQASHDISKYLNWYQQKPGKAPKLLIYDASNLETGVPSRFSGSRSGTDFTLTISSLQPEDFATYYCQQXYTTPPTFGQGTKLEI

SEQ ID NO: 88 - protein, 106 aa, synthetic construct
  SITE 91: note = natural amino acid or unnatural amino acid
DIQMTQSPSSLSASVGDRVTITCRATQAISNYLAWYQQKPGKAPKLLIYDVSNVQTGVPSRFSGSRSGTDFTLTISSLQPEDFATYYCQQXYTTPPTFGQGTKLEI

SEQ ID NO: 89 - protein, 106 aa, synthetic construct
  SITE 91: note = natural amino acid or unnatural amino acid
DIQMTQSPSSLSASVGDRVTITCRTSQGITDPLNWYQQKPGKAPKLLIYKTSSLESGVPSRFSGSRSGTDFTLTISSLQPEDFATYYCQQXYTTPPTFGQGTKLEI

SEQ ID NO: 90 - protein, 106 aa, synthetic construct
  SITE 91: note = natural amino acid or unnatural amino acid
DIQMTQSPSSLSASVGDRVTITCRASQGLSSWLAWYQQKPGKAPKLLIYDASNLETGVPSRFSGSRSGTDFTLTISSLQPEDFATYYCQQXYTTPPTFGQGTKLEI

SEQ ID NO: 91 - protein, 106 aa, synthetic construct
  SITE 91: note = natural amino acid or unnatural amino acid
DIQMTQSPSSLSASVGDRVTITCRASQNIGTYLAWYQQKPGKAPKLLIYDASNLETGVPSRFSGSRSGTDFTLTISSLQPEDFATYYCQQXYTTPPTFGQGTKLEI

SEQ ID NO: 92 - protein, 106 aa, synthetic construct
  SITE 91: note = natural amino acid or unnatural amino acid
DIQMTQSPSSLSASVGDRVTITCQASQDISNYLNWYQQKPGKAPNLLIYAASTLQSGVPSRFSGSRSGTDFTLTISSLQPEDFATYYCQQXYTTPPTFGQGTKLEI

SEQ ID NO: 93 - protein, 11 aa, synthetic construct
RASQVIGNDLG

SEQ ID NO: 94 - protein, 11 aa, synthetic construct
RASQYISTYLN

SEQ ID NO: 95 - protein, 11 aa, synthetic construct
RASQSISSWLA

SEQ ID NO: 96 - protein, 11 aa, synthetic construct
QASQDIRNDLN

SEQ ID NO: 97 - protein, 11 aa, synthetic construct
RASQGISSDLG

SEQ ID NO: 98 - protein, 14 aa, synthetic construct
AMGPSSGAPGGGGS

SEQ ID NO: 99 - protein, 11 aa, synthetic construct
RASQSIGSSLH

SEQ ID NO: 100 - protein, 11 aa, synthetic construct
QASQDISNSLN

SEQ ID NO: 101 - protein, 16 aa, synthetic construct
KLLIYDVSNVQTGVPS

SEQ ID NO: 102 - protein, 16 aa, synthetic construct
KVLISKTSYLESGVPS

SEQ ID NO: 103 - protein, 16 aa, synthetic construct
NLLMYAASSLQSGVPS

SEQ ID NO: 104 - protein, 16 aa, synthetic construct
KSLIYAASRLQSGVPS

SEQ ID NO: 105 - protein, 16 aa, synthetic construct
KLLIYDASSLESGVPS

SEQ ID NO: 106 - protein, 12 aa, synthetic construct
GGASPAAPAPAG

SEQ ID NO: 107 - protein, 16 aa, synthetic construct
TVLIYAASSLQTGVPS

SEQ ID NO: 108 - protein, 16 aa, synthetic construct
NLLIYATSNLQSGVPS

SEQ ID NO: 109 - protein, 9 aa, synthetic construct
FTFSGHWMH

SEQ ID NO: 110 - protein, 9 aa, synthetic construct
FTFSASYMS

SEQ ID NO: 111 - protein, 9 aa, synthetic construct
FTFSDYWIS

SEQ ID NO: 112 - protein, 9 aa, synthetic construct
FTFSKFWMH

SEQ ID NO: 113 - protein, 8 aa, synthetic construct
GGASPAGG

SEQ ID NO: 114 - protein, 9 aa, synthetic construct
FPFSGHWMH

SEQ ID NO: 115 - protein, 22 aa, synthetic construct
WVASISDSSSYIYYADSVRGRF

SEQ ID NO: 116 - protein, 21 aa, synthetic construct
WIGSIYYSGSTYYNPSLKSRV

SEQ ID NO: 117 - protein, 21 aa, synthetic construct
WIGNVYYSGNAYYNPSLESRV

SEQ ID NO: 118 - protein, 22 aa, synthetic construct
WVSGISGSGGSTYYADSVKGRF

SEQ ID NO: 119 - protein, 22 aa, synthetic construct
WVSAISGSGGSTYYADSVKGRF

SEQ ID NO: 120 - protein, 22 aa, synthetic construct
WVSSISSSSSYIYYADSVKGRF

SEQ ID NO: 121 - protein, 5 aa, synthetic construct
GSPAG

SEQ ID NO: 122 - protein, 22 aa, synthetic construct
WVSGISGTGATSHYADSVKGRF

SEQ ID NO: 123 - protein, 22 aa, synthetic construct
WVSAISGSGGSTYYADSVKGRF

SEQ ID NO: 124 - protein, 13 aa, synthetic construct
ARDYEGATRAADY

SEQ ID NO: 125 - protein, 13 aa, synthetic construct
ARGAPYYEGAFDI

SEQ ID NO: 126 - protein, 11 aa, synthetic construct
ARNTGFETLDN

SEQ ID NO: 127 - protein, 15 aa, synthetic construct
ARELTMATTTDAFDI

SEQ ID NO: 128 - protein, 16 aa, synthetic construct
AREVTMVRGVTDAFDI

SEQ ID NO: 129 - protein, 12 aa, synthetic construct
ARDPISTGAFDI

SEQ ID NO: 130 - protein, 10 aa, synthetic construct
PKPSTPPGSS

SEQ ID NO: 131 - protein, 15 aa, synthetic construct
AREVITAASTDAFDL

SEQ ID NO: 132 - protein, 15 aa, synthetic construct
ARELTMASTTDAFDF

SEQ ID NO: 133 - protein, 106 aa, synthetic construct
  SITE 91: note = natural amino acid or unnatural amino acid
DIQMTQSPSSLSASVGDRVTITCRASQVIGNDLGWYQQKPGKAPKLLIYDVSNVQTGVPSRFSGSRSGTDFTLTISSLQPEDFATYYCQQXYTTPPTFGQGTKLEI

SEQ ID NO: 134 - protein, 106 aa, synthetic construct
  SITE 91: note = natural amino acid or unnatural amino acid
DIQMTQSPSSLSASVGDRVTITCRASQYISTYLNWYQQKPGKAPKVLISKTSYLESGVPSRFSGSRSGTDFTLTISSLQPEDFATYYCQQXYTTPPTFGQGTKLEI

SEQ ID NO: 135 - protein, 106 aa, synthetic construct
  SITE 91: note = natural amino acid or unnatural amino acid
DIQMTQSPSSLSASVGDRVTITCRASQSISSWLAWYQQKPGKAPNLLMYAASSLQSGVPSRFSGSRSGTDFTLTISSLQPEDFATYYCQQXYTTPPTFGQGTKLEI

SEQ ID NO: 136 - protein, 106 aa, synthetic construct
  SITE 91: note = natural amino acid or unnatural amino acid
DIQMTQSPSSLSASVGDRVTITCQASQDIRNDLNWYQQKPGKAPKSLIYAASRLQSGVPSRFSGSRSGTDFTLTISSLQPEDFATYYCQQXYTTPPTFGQGTKLEI

SEQ ID NO: 137 - protein, 106 aa, synthetic construct
  SITE 91: note = natural amino acid or unnatural amino acid
DIQMTQSPSSLSASVGDRVTITCRASQGISSDLGWYQQKPGKAPKLLIYDVSNVQTGVPSRFSGSRSGTDFTLTISSLQPEDFATYYCQQXYTTPPTFGQGTKLEI

SEQ ID NO: 138 - protein, 106 aa, synthetic construct
  SITE 91: note = natural amino acid or unnatural amino acid
DIQMTQSPSSLSASVGDRVTITCRASQSISSWLAWYQQKPGKAPKLLIYDASSLESGVPSRFSGSRSGTDFTLTISSLQPEDFATYYCQQXYTTPPTFGQGTKLEI

SEQ ID NO: 139 - protein, 11 aa, synthetic construct
KLYPYDVPDYA

SEQ ID NO: 140 - protein, 106 aa, synthetic construct
  SITE 91: note = natural amino acid or unnatural amino acid
DIQMTQSPSSLSASVGDRVTITCRASQSIGSSLHWYQQKPGKAPTVLIYAASSLQTGVPSRFSGSRSGTDFTLTISSLQPEDFATYYCQQXYTTPPTFGQGTKLEI

SEQ ID NO: 141 - protein, 106 aa, synthetic construct
  SITE 91: note = natural amino acid or unnatural amino acid
DIQMTQSPSSLSASVGDRVTITCQASQDISNSLNWYQQKPGKAPNLLIYATSNLQSGVPSRFSGSRSGTDFTLTISSLQPEDFATYYCQQXYTTPPTFGQGTKLEI

SEQ ID NO: 142 - protein, 120 aa, synthetic construct
EVQLVESGGGLVQPGGSLRLSCAASGFTFSGHWMHWVRQAPGKGLEWVASISDSSSYIYYADSVRGRFTISRDNAKKTLYLQMNSLRAEDTAVYYCARDYEGATRAADYWGQGTLVTVSS

SEQ ID NO: 143 - protein, 119 aa, synthetic construct
EVQLVESGGGLVQPGGSLRLSCAASGFTFSASYMSWVRQAPGKGLEWIGSIYYSGSTYYNPSLKSRVTISADTSKNTAYLQMNSLRAEDTAVYYCARGAPYYEGAFDIWGQGTLVTVSS

SEQ ID NO: 144 - protein, 117 aa, synthetic construct
EVQLVESGGGLVQPGGSLRLSCAASGFTFSDYWISWVRQAPGKGLEWIGNVYYSGNAYYNPSLESRVTISADTSKNTAYLQMNSLRAEDTAVYYCARNTGFETLDNWGQGTLVTVSS

SEQ ID NO: 145 - protein, 122 aa, synthetic construct
EVQLVESGGGLVQPGGSLRLSCAASGFTFSGHWMHWVRQAPGKGLEWVSGISGSGGSTYYADSVKGRFTISADTSKNTAYLQMNSLRAEDTAVYYCARELTMATTTDAFDIWGQGTLVTVSS

SEQ ID NO: 146 - protein, 123 aa, synthetic construct
EVQLVESGGGLVQPGGSLRLSCAASGFTFSGHWMHWVRQAPGKGLEWVSAISGSGGSTYYADSVKGRFTISADTSKNTAYLQMNSLRAEDTAVYYCAREVTMVRGVTDAFDIWGQGTLVTVSS

SEQ ID NO: 147 - protein, 119 aa, synthetic construct
EVQLVESGGGLVQPGGSLRLSCAASGFTFSKFWMHWVRQAPGKGLEWVSSISSSSSYIYYADSVKGRFTISADTSKNTAYLQMNSLRAEDTAVYYCARDPISTGAFDIWGQGTLVTVSS

SEQ ID NO: 148 - protein, 16 aa, synthetic construct
EEEEKKKKEEEEKKKK

SEQ ID NO: 149 - protein, 122 aa, synthetic construct
EVQLVESGGGLVQPGGSLRLSCAASGFPFSGHWMHWVRQAPGKGLEWVSGISGTGATSHYADSVKGRFTISADTSKNTAYLQMNSLRAEDTAVYYCAREVITAASTDAFDLWGQGTLVTVSS

SEQ ID NO: 150 - protein, 122 aa, synthetic construct
EVQLVESGGGLVQPGGSLRLSCAASGFTFSGHWMHWVRQAPGKGLEWVSAISGSGGSTYYADSVKGRFTISADTSKNTAYLQMNSLRAEDTAVYYCARELTMASTTDAFDFWGQGTLVTVSS

SEQ ID NO: 151 - protein, 11 aa, synthetic construct
QASQGISHALA

SEQ ID NO: 152 - protein, 11 aa, synthetic construct
RASQTISDWLA

SEQ ID NO: 153 - protein, 11 aa, synthetic construct
RASQSISSDLN

SEQ ID NO: 154 - protein, 11 aa, synthetic construct
QASQDISNYLN

SEQ ID NO: 155 - protein, 11 aa, synthetic construct
RTSQSVNNHLN

SEQ ID NO: 156 - protein, 11 aa, synthetic construct
RASQPISDWLA

SEQ ID NO: 157 - protein, 16 aa, synthetic construct
KLLIYAASSLQSGVPS

SEQ ID NO: 158 - protein, 16 aa, synthetic construct
KLLIYDASSLESGVPS

SEQ ID NO: 159 - protein, 16 aa, synthetic construct
KLLIYRATFLESGVPS

SEQ ID NO: 160 - protein, 16 aa, synthetic construct
KLLIYAASRLQSGVPS

SEQ ID NO: 161 - protein, 16 aa, synthetic construct
NLLMYAASSLQSGVPS

SEQ ID NO: 162 - protein, 16 aa, synthetic construct
KLLIYRASSLESGVPS

SEQ ID NO: 163 - protein, 16 aa, synthetic construct
KSLIYDAYNLQSGVPP

SEQ ID NO: 164 - protein, 9 aa, synthetic construct
FTFSTYVMH

SEQ ID NO: 165 - protein, 9 aa, synthetic construct
FTFSDYAMT

SEQ ID NO: 166 - protein, 9 aa, synthetic construct
FTFSSYCMN

SEQ ID NO: 167 - protein, 9 aa, synthetic construct
FSFSKFWMH

SEQ ID NO: 168 - protein, 9 aa, synthetic construct
FTFSNFAMH

SEQ ID NO: 169 - protein, 9 aa, synthetic construct
FTFSSFSMS

SEQ ID NO: 170 - protein, 9 aa, synthetic construct
FTFSGHWMH

SEQ ID NO: 171 - protein, 22 aa, synthetic construct
WLANIDTGGGVTNYADSVKGRF

SEQ ID NO: 172 - protein, 23 aa, synthetic construct
VWVSRIKHDGSSTAYADSVKGRF

SEQ ID NO: 173 - protein, 22 aa, synthetic construct
WVSSVTGSAQRTNYADSVKGRF

SEQ ID NO: 174 - protein, 22 aa, synthetic construct
WVAFMAHDESNKNYADSVKGRF

SEQ ID NO: 175 - protein, 23 aa, synthetic construct
YVSAISGGNGGGTYYADSAKGRF

SEQ ID NO: 176 - protein, 22 aa, synthetic construct
WVANIKEDGSDKYYVDSVTGRF

SEQ ID NO: 177 - protein, 22 aa, synthetic construct
WVAVISSDGSYKSYADSVKGRF

SEQ ID NO: 178 - protein, 11 aa, synthetic construct
ARNSGFETLDY

SEQ ID NO: 179 - protein, 10 aa, synthetic construct
AREGNYCLDY

SEQ ID NO: 180 - protein, 11 aa, synthetic construct
ARDKVCNTFDI

SEQ ID NO: 181 - protein, 10 aa, synthetic construct
AREGNYCLDY

SEQ ID NO: 182 - protein, 12 aa, synthetic construct
ARDWGAAAVLHH

SEQ ID NO: 183 - protein, 11 aa, synthetic construct
ASRTVAGTLDY

SEQ ID NO: 184 - protein, 106 aa, synthetic construct
  SITE 91: note = natural amino acid or unnatural amino acid
DIQMTQSPSSLSASVGDRVTITCQASQGISHALAWYQQKPGKAPKLLIYAASSLQSGVPSRFSGSRSGTDFTLTISSLQPEDFATYYCQQXYTTPPTFGQGTKLEI

SEQ ID NO: 185 - protein, 106 aa, synthetic construct
  SITE 91: note = natural amino acid or unnatural amino acid
DIQMTQSPSSLSASVGDRVTITCRASQTISDWLAWYQQKPGKAPKLLIYDASSLESGVPSRFSGSRSGTDFTLTISSLQPEDFATYYCQQXYTTPPTFGQGTKLEI

SEQ ID NO: 186 - protein, 106 aa, synthetic construct
  SITE 91: note = natural amino acid or unnatural amino acid
DIQMTQSPSSLSASVGDRVTITCRASQSISSDLNWYQQKPGKAPKLLIYRATFLESGVPSRFSGSRSGTDFTLTISSLQPEDFATYYCQQXYTTPPTFGQGTKLEI

SEQ ID NO: 187 - protein, 106 aa, synthetic construct
  SITE 91: note = natural amino acid or unnatural amino acid
DIQMTQSPSSLSASVGDRVTITCQASQDISNYLNWYQQKPGKAPKLLIYAASRLQSGVPSRFSGSRSGTDFTLTISSLQPEDFATYYCQQXYTTPPTFGQGTKLEI

SEQ ID NO: 188 - protein, 106 aa, synthetic construct
  SITE 91: note = natural amino acid or unnatural amino acid
DIQMTQSPSSLSASVGDRVTITCRASQPISDWLAWYQQKPGKAPKSLIYDAYNLQSGVPPRFSGSRSGTDFTLTISSLQPEDFATYYCQQXYTTPPTFGQGTKLEI

SEQ ID NO: 189 - protein, 106 aa, synthetic construct
  SITE 91: note = natural amino acid or unnatural amino acid
DIQMTQSPSSLSASVGDRVTITCRTSQSVNNHLNWYQQKPGKAPKLLIYRASSLESGVPSRFSGSRSGTDFTLTISSLQPEDFATYYCQQXYTTPPTFGQGTKLEI

SEQ ID NO: 190 - protein, 106 aa, synthetic construct; identical to SEQ ID NO: 135
  SITE 91: note = natural amino acid or unnatural amino acid

SEQ ID NO: 191 - protein, 118 aa, synthetic construct
EVQLVESGGGLVQPGGSLRLSCAASGFTFSTYVMHWVRQAPGKGLEWLANIDTGGGVTNYADSVKGRFTISADTSKNTAYLQMNSLRAEDTAVYYCARNSGFETLDYWGQGTLVTVSS

SEQ ID NO: 192 - protein, 117 aa, synthetic construct
EVQLVESGGGLVQPGGSLRLSCAASGFTFSDYAMTWVRQAPGKGLVWVSRIKHDGSSTAYADSVKGRFTISADTSKNTAYLQMNSLRAEDTAVYYCAREGNYCLDYWGQGTLVTVSS

SEQ ID NO: 193 - protein, 118 aa, synthetic construct
EVQLVESGGGLVQPGGSLRLSCAASGFTFSSYCMNWVRQAPGKGLEWVSSVTGSAQRTNYADSVKGRFTISADTSKNTAYLQMNSLRAEDTAVYYCARNTGFETLDNWGQGTLVTVSS

SEQ ID NO: 194 - protein, 118 aa, synthetic construct
EVQLVESGGGLVQPGGSLRLSCAASGFSFSKFWMHWVRQAPGKGLEWVAFMAHDESNKNYADSVKGRFTISADTSKNTAYLQMNSLRAEDTAVYYCARDKVCNTFDIWGQGTLVTVSS

SEQ ID NO: 195 - protein, 118 aa, synthetic construct
EVQLVESGGGLVQPGGSLRLSCAASGFTFSNFAMHWVRQAPGKGLEYVSAISGGNGGGTYYADSAKGRFTISADTSKNTAYLQMNSLRAEDTAVYYCAREGNYCLDYWGQGTLVTVSS

SEQ ID NO: 196 - protein, 119 aa, synthetic construct
EVQLVESGGGLVQPGGSLRLSCAASGFTFSSFSMSWVRQAPGKGLEWVANIKEDGSDKYYVDSVTGRFTISADTSKNTAYLQMNSLRAEDTAVYYCARDWGAAAVLHHWGQGTLVTVSS

SEQ ID NO: 197 - protein, 118 aa, synthetic construct
EVQLVESGGGLVQPGGSLRLSCAASGFTFSGHWMHWVRQAPGKGLEWVAVISSDGSYKSYADSVKGRFTISADTSKNTAYLQMNSLRAEDTAVYYCASRTVAGTLDYWGQGTLVTVSS

SEQ ID NO: 198 - protein, 11 aa, synthetic construct
QASQDISHYLN

SEQ ID NO: 199 - protein, 11 aa, synthetic construct
RASQGISSDLG

SEQ ID NO: 200 - protein, 11 aa, synthetic construct
RASETIGSWLA

SEQ ID NO: 201 - protein, 11 aa, synthetic construct
RASQNINRHLN

SEQ ID NO: 202 - protein, 11 aa, synthetic construct
QASQDIGKFLN

SEQ ID NO: 203 - protein, 11 aa, synthetic construct
RASQSISDWLA

SEQ ID NO: 204 - protein, 16 aa, synthetic construct
KLLIHRVSSLESGVPS

SEQ ID NO: 205 - protein, 16 aa, synthetic construct
KLLIYDVSNVQTGVPS

SEQ ID NO: 206 - protein, 16 aa, synthetic construct
KLLIYKSTTVEGGVSS

SEQ ID NO: 207 - protein, 16 aa, synthetic construct
KLLIYDVSNVQTGVPS

SEQ ID NO: 208 - protein, 16 aa, synthetic construct
KLLISATSNLQWGVPS

SEQ ID NO: 209 - protein, 16 aa, synthetic construct
KLLIYAASSLQSGVPS

SEQ ID NO: 210 - protein, 9 aa, synthetic construct
FSFSTYAMH

SEQ ID NO: 211 - protein, 9 aa, synthetic construct
FTFSGHWMH

SEQ ID NO: 212 - protein, 9 aa, synthetic construct
FTFTSYAMA

SEQ ID NO: 213 - protein, 9 aa, synthetic construct
FTFDEYIMH

SEQ ID NO: 214 - protein, 9 aa, synthetic construct
FSFSNFAMT

SEQ ID NO: 215 - protein, 9 aa, synthetic construct
FPFSGHWMH

SEQ ID NO: 216 - protein, 22 aa, synthetic construct
WVANIDGDGGVTNYAGSVKGRF

SEQ ID NO: 217 - protein, 22 aa, synthetic construct
WVSAISGSGGSTYYADSVKGRF

SEQ ID NO: 218 - protein, 22 aa, synthetic construct
WVSSISNGGSVIYYANSVKGRF

SEQ ID NO: 219 - protein, 22 aa, synthetic construct
YVSAISSNGGSTYYANSVKGRF

SEQ ID NO: 220 - protein, 22 aa, synthetic construct
WVSSISNGGSVIYYANSVKGRF

SEQ ID NO: 221 - protein, 22 aa, synthetic construct
WVSGISWNGGTTGYADSVKGRF

SEQ ID NO: 222 - protein, 11 aa, synthetic construct
ARDRGWLQFDY

SEQ ID NO: 223 - protein, 16 aa, synthetic construct
AREVTMVRGVTDAFDI

SEQ ID NO: 224 - protein, 11 aa, synthetic construct
ARDRGFLQFDY

SEQ ID NO: 225 - protein, 11 aa, synthetic construct
ARDRGFLQFDY

SEQ ID NO: 226 - protein, 11 aa, synthetic construct
ARDRGFLQFDY

SEQ ID NO: 227 - protein, 12 aa, synthetic construct
ARDDYGGDSFDS

SEQ ID NO: 228 - protein, 106 aa, synthetic construct
  SITE 91: note = natural amino acid or unnatural amino acid
DIQMTQSPSSLSASVGDRVTITCQASQDISHYLNWYQQKPGKAPKLLIHRVSSLESGVPSRFSGSRSGTDFTLTISSLQPEDFATYYCQQXYTTPPTFGQGTKLEI

SEQ ID NO: 229 - protein, 106 aa, synthetic construct; identical to SEQ ID NO: 137
  SITE 91: note = natural amino acid or unnatural amino acid

SEQ ID NO: 230 - protein, 106 aa, synthetic construct
  SITE 91: note = natural amino acid or unnatural amino acid
DIQMTQSPSSLSASVGDRVTITCRASETIGSWLAWYQQKPGKAPKLLIYKSTTVEGGVSSRFSGSRSGTDFTLTISSLQPEDFATYYCQQXYTTPPTFGQGTKLEI

SEQ ID NO: 231 - protein, 106 aa, synthetic construct
  SITE 91: note = natural amino acid or unnatural amino acid
DIQMTQSPSSLSASVGDRVTITCRASQNINRHLNWYQQKPGKAPKLLIYDVSNVQTGVPSRFSGSRSGTDFTLTISSLQPEDFATYYCQQXYTTPPTFGQGTKLEI

SEQ ID NO: 232 - protein, 106 aa, synthetic construct
  SITE 91: note = natural amino acid or unnatural amino acid
DIQMTQSPSSLSASVGDRVTITCQASQDIGKFLNWYQQKPGKAPKLLISATSNLQWGVPSRFSGSRSGTDFTLTISSLQPEDFATYYCQQXYTTPPTFGQGTKLEI

SEQ ID NO: 233 - protein, 106 aa, synthetic construct
  SITE 91: note = natural amino acid or unnatural amino acid
DIQMTQSPSSLSASVGDRVTITCRASQSISDWLAWYQQKPGKAPKLLIYAASSLQSGVPSRFSGSRSGTDFTLTISSLQPEDFATYYCQQXYTTPPTFGQGTKLEI

SEQ ID NO: 234 - protein, 118 aa, synthetic construct
EVQLVESGGGLVQPGGSLRLSCAASGFSFSTYAMHWVRQAPGKGLEWVANIDGDGGVTNYAGSVKGRFTISADTSKNTAYLQMNSLRAEDTAVYYCARDRGWLQFDYWGQGTLVTVSS

SEQ ID NO: 235 - protein, 123 aa, synthetic construct; identical to SEQ ID NO: 146

SEQ ID NO: 236 - protein, 118 aa, synthetic construct
EVQLVESGGGLVQPGGSLRLSCAASGFTFTSYAMAWVRQAPGKGLEWVSSISNGGSVIYYANSVKGRFTISRDNSKKTLYLQMNGLRVEDTAVYYCARDRGFLQFDYWGQGTLVTVSS

SEQ ID NO: 237 - protein, 118 aa, synthetic construct
EVQLVESGGGLVQPGGSLRLSCAASGFTFDEYIMHWVRQAPGKGLEYVSAISSNGGSTYYANSVKGRFTISADTSKNTAYLQMNSLRAEDTAVYYCARDRGFLQFDYWGQGTLVTVSS

SEQ ID NO: 238 - protein, 118 aa, synthetic construct
EVQLVESGGGLVQPGGSLRLSCAASGFSFSNFAMTWVRQAPGKGLEWVSSISNGGSVIYYANSVKGRFTISRDNSKKTLYLQMNSLRAEDTAVYYCARDRGFLQFDYWGQGTLVTVSS

SEQ ID NO: 239 - protein, 119 aa, synthetic construct
EVQLVESGGGLVQPGGSLRLSCAASGFPFSGHWMHWVRQAPGKGLEWVSGISWNGGTTGYADSVKGRFTISRDNAKNSVYLQMNSLRAEDTAVYYCARDDYGGDSFDSWGQGTLVTVSS

SEQ ID NO: 240 - protein, 15 aa, synthetic construct
LLTPPPPPLFPPPFF

SEQ ID NO: 241 - protein, 10 aa, synthetic construct
EAAAKEAAAK

SEQ ID NO: 242 - protein, 15 aa, synthetic construct
EAAAKEAAAKEAAAK

SEQ ID NO: 243 - protein, 20 aa, synthetic construct
EAAAKEAAAKEAAAKEAAAK

SEQ ID NO: 244 - protein, 25 aa, synthetic construct
EAAAKEAAAKEAAAKEAAAKEAAAK

SEQ ID NO: 245 - protein, 8 aa, synthetic construct
EEEEKKKK

SEQ ID NO: 246 - protein, 16 aa, synthetic construct
EEEERRRREEEERRRR

SEQ ID NO: 247 - protein, 11 aa, synthetic construct
QASQDIRNSLN

SEQ ID NO: 248 - protein, 11 aa, synthetic construct
RASQSISRALA

SEQ ID NO: 249 - protein, 11 aa, synthetic construct
QASQSISRYLS

SEQ ID NO: 250 - protein, 11 aa, synthetic construct
RASQNIGTSLH

SEQ ID NO: 251 - protein, 16 aa, synthetic construct
KLLIKYASQSISGVPS

SEQ ID NO: 252 - protein, 16 aa, synthetic construct
KLLIYKASSLQSGVPS

SEQ ID NO: 253 - protein, 16 aa, synthetic construct
KLLIYKTSRLESGVPS

SEQ ID NO: 254 - protein, 16 aa, synthetic construct
KLLIYAASTLQSGVPS

SEQ ID NO: 255 - protein, 16 aa, synthetic construct
KLLISRASSLQSGVPS

SEQ ID NO: 256 - protein, 9 aa, synthetic construct
FTFSGHWMH

SEQ ID NO: 257 - protein, 9 aa, synthetic construct
FTVGSNSMT

SEQ ID NO: 258 - protein, 9 aa, synthetic construct
FTFGSFWMS

SEQ ID NO: 259 - protein, 9 aa, synthetic construct
FRFSSYSMN

SEQ ID NO: 260 - protein, 9 aa, synthetic construct
FTFSNHAMH

SEQ ID NO: 261 - protein, 21 aa, synthetic construct
WIGTVSYNGRTYYNPSLKSRV

SEQ ID NO: 262 - protein, 22 aa, synthetic construct
WVSSISGTGGRTYYADSVKGRF

SEQ ID NO: 263 - protein, 22 aa, synthetic construct
WVSSITGDSNYRYYADSVKGRF

SEQ ID NO: 264 - protein, 22 aa, synthetic construct
WVSSISNGGSVIYYANSVKGRF

SEQ ID NO: 265 - protein, 22 aa, synthetic construct
WVSGISGSGGSTYYADPVKGRF

SEQ ID NO: 266 - protein, 22 aa, synthetic construct
WVSAITGNGRSKYYADSVKGRF

SEQ ID NO: 267 - protein, 15 aa, synthetic construct
ARGASGRTYNNFFDP

SEQ ID NO: 268 - protein, 21 aa, synthetic construct
ARILPVRGASGQWARKNWFDP

SEQ ID NO: 269 - protein, 13 aa, synthetic construct
ARDRSGSLRAFDY

SEQ ID NO: 270 - protein, 13 aa, synthetic construct
ARGLRRASGPFDY

SEQ ID NO: 271 - protein, 13 aa, synthetic construct
ARGGRGPTTPFDY

SEQ ID NO: 272 - protein, 11 aa, synthetic construct
ARDRGWLQFDY

SEQ ID NO: 273 - protein, 121 aa, synthetic construct
EVQLVESGGGLVQPGGSLRLSCAASGFTFSGHWMHWVRQAPGKGLEWIGTVSYNGRTYYNPSLKSRVTISADTSKNTAYLQMNSLRAEDTAVYYCARGASGRTYNNFFDPWGQGTLVTVSS

SEQ ID NO: 274 - protein, 128 aa, synthetic construct
EVQLVESGGGLVQPGGSLRLSCAASGFTVGSNSMTWVRQAPGKGLEWVSSISGTGGRTYYADSVKGRFTISADTSKNTAYLQMNSLRAEDTAVYYCARILPVRGASGQWARKNWFDPWGQGTLVTVSS

SEQ ID NO: 275 - protein, 120 aa, synthetic construct
EVQLVESGGGLVQPGGSLRLSCAASGFTFSGHWMHWVRQAPGKGLEWVSSITGDSNYRYYADSVKGRFTISADTSKNTAYLQMNSLRAEDTAVYYCARDRSGSLRAFDYWGQGTLVTVSS

SEQ ID NO: 276 - protein, 120 aa, synthetic construct
EVQLVESGGGLVQPGGSLRLSCAASGFTFGSFWMSWVRQAPGKGLEWVSSISNGGSVIYYANSVKGRFTISRDNSKKTLYLQMNSLRAEDTAVYYCARGLRRASGPFDYWGQGTLVTVSS

SEQ ID NO: 277 - protein, 120 aa, synthetic construct
EVQLVESGGGLVQPGGSLRLSCAASGFRFSSYSMNWVRQAPGKGLEWVSGISGSGGSTYYADPVKGRFTISADTSKNTAYLQMNSLRAEDTAVYYCARGGRGPTTPFDYWGQGTLVTVSS

SEQ ID NO: 278 - protein, 118 aa, synthetic construct
EVQLVESGGGLVQPGGSLRLSCAASGFTFSNHAMHWVRQAPGKGLEWVSAITGNGRSKYYADSVKGRFTISADTSKNTAYLQMNSLRAEDTAVYYCARDRGWLQFDYWGQGTLVTVSS

SEQ ID NO: 279 - protein, 106 aa, synthetic construct
  SITE 91: note = natural amino acid or unnatural amino acid
DIQMTQSPSSLSASVGDRVTITCQASQDIRNSLNWYQQKPGKAPKLLIKYASQSISGVPSRFSGSRSGTDFTLTISSLQPEDFATYYCQQXYTTPPTFGQGTKLEI

SEQ ID NO: 280 - protein, 106 aa, synthetic construct
  SITE 91: note = natural amino acid or unnatural amino acid
DIQMTQSPSSLSASVGDRVTITCRASQSISRALAWYQQKPGKAPKLLIYKASSLQSGVPSRFSGSRSGTDFTLTISSLQPEDFATYYCQQXYTTPPTFGQGTKLEI

SEQ ID NO: 281 - protein, 106 aa, synthetic construct
  SITE 91: note = natural amino acid or unnatural amino acid
DIQMTQSPSSLSASVGDRVTITCQASQSISRYLSWYQQKPGKAPKLLIYKTSRLESGVPSRFSGSRSGTDFTLTISSLQPEDFATYYCQQXYTTPPTFGQGTKLEI

SEQ ID NO: 282 - protein, 106 aa, synthetic construct
  SITE 91: note = natural amino acid or unnatural amino acid
DIQMTQSPSSLSASVGDRVTITCQASQDIRNSLNWYQQKPGKAPKLLIYAASTLQSGVPSRFSGSRSGTDFTLTISSLQPEDFATYYCQQXYTTPPTFGQGTKLEI

SEQ ID NO: 283 - protein, 106 aa, synthetic construct
  SITE 91: note = natural amino acid or unnatural amino acid
DIQMTQSPSSLSASVGDRVTITCRASQNIGTSLHWYQQKPGKAPKLLISRASSLQSGVPSRFSGSRSGTDFTLTISSLQPEDFATYYCQQXYTTPPTFGQGTKLEI

SEQ ID NO: 284 - protein, 16 aa, synthetic construct
KLLIYKTSNLESGVPS

SEQ ID NO: 285 - protein, 106 aa, synthetic construct
  SITE 91: note = natural amino acid or unnatural amino acid
DIQMTQSPSSLSASVGDRVTITCRASQSISSWLAWYQQKPGKAPKLLIYKTSNLESGVPSRFSGSRSGTDFTLTISSLQPEDFATYYCQQXYTTPPTFGQGTKLEI